European Patent Application EP 4 803 536 A1, published September 9, 2026. Title: NOVEL FUSIONS PROTEINS FOR EXTENDED HALF-LIFE OF VEGF BINDING PROTEINS. Applicant: Navigo Proteins GmbH. Application EP. The sequence listing filed with the application follows.

SEQUENCE LISTING (8 sequences)

SEQ ID NO: 1 - protein, 44 aa, synthetic construct
LAEAKVLALKELDKYGISNYYKNLINNAKTVEGVKALKEAIVAA

SEQ ID NO: 2 - protein, 46 aa, synthetic construct
LAEAKVLALKELDKYGISNYYKNLINNAKTVEGVKALKEAIVAALP

SEQ ID NO: 3 - protein, 431 aa, synthetic construct
SDTGRPFVEMYSEIPEIIHMTEGRELVIPCRVTSPNITVTLKKFPLDTLIPDGKRIIWDSRKGFIISNATYKEIGLLTCEATVNGHLYKTNYLTHRQTNTIIDVVLSPSHGIELSVGEKLVLNCTARTELNVGIDFNWEYPSSKHQHKKLVNRDLKTQSGSEMKKFLSTLTIDGVTRSDQGLYTCAASSGLMTKKNSTFVRVHEKDKTHTCPPCPAPELLGGPSVFLFPPKPKDTLMISRTPEVTCVVVDVSHEDPEVKFNWYVDGVEVHNAKTKPREEQYNSTYRVVSVLTVLHQDWLNGKEYKCKVSNKALPAPIEKTISKAKGQPREPQVYTLPPSRDELTKNQVSLTCLVKGFYPSDIAVEWESNGQPENNYKTTPPVLDSDGSFFLYSKLTVDKSRWQQGNVFSCSVMHEALHNHYTQKSLSLSPG

SEQ ID NO: 4 - protein, 548 aa, synthetic construct
  source 1..548: note = Fusion protein 229658
SDTGRPFVEMYSEIPEIIHMTEGRELVIPCRVTSPNITVTLKKFPLDTLIPDGKRIIWDSRKGFIISNATYKEIGLLTCEATVNGHLYKTNYLTHRQTNTIIDVVLSPSHGIELSVGEKLVLNCTARTELNVGIDFNWEYPSSKHQHKKLVNRDLKTQSGSEMKKFLSTLTIDGVTRSDQGLYTCAASSGLMTKKNSTFVRVHEKDKTHTCPPCPAPELLGGPSVFLFPPKPKDTLMISRTPEVTCVVVDVSHEDPEVKFNWYVDGVEVHNAKTKPREEQYNSTYRVVSVLTVLHQDWLNGKEYKCKVSNKALPAPIEKTISKAKGQPREPQVYTLPPSRDELTKNQVSLTCLVKGFYPSDIAVEWESNGQPENNYKTTPPVLDSDGSFFLYSKLTVDKSRWQQGNVFSCSVMHEALHNHYTQKSLSLSPGGGGGSGGGGSGGGGSLAEAKVLALKELDKYGISNYYKNLINNAKTVEGVKALKEAIVAALPGGGGSGGGGSLAEAKVLALKELDKYGISNYYKNLINNAKTVEGVKALKEAIVAALP

SEQ ID NO: 5 - protein, 492 aa, synthetic construct
  source 1..492: note = Fusion protein 229657
SDTGRPFVEMYSEIPEIIHMTEGRELVIPCRVTSPNITVTLKKFPLDTLIPDGKRIIWDSRKGFIISNATYKEIGLLTCEATVNGHLYKTNYLTHRQTNTIIDVVLSPSHGIELSVGEKLVLNCTARTELNVGIDFNWEYPSSKHQHKKLVNRDLKTQSGSEMKKFLSTLTIDGVTRSDQGLYTCAASSGLMTKKNSTFVRVHEKDKTHTCPPCPAPELLGGPSVFLFPPKPKDTLMISRTPEVTCVVVDVSHEDPEVKFNWYVDGVEVHNAKTKPREEQYNSTYRVVSVLTVLHQDWLNGKEYKCKVSNKALPAPIEKTISKAKGQPREPQVYTLPPSRDELTKNQVSLTCLVKGFYPSDIAVEWESNGQPENNYKTTPPVLDSDGSFFLYSKLTVDKSRWQQGNVFSCSVMHEALHNHYTQKSLSLSPGGGGGSGGGGSGGGGSLAEAKVLALKELDKYGISNYYKNLINNAKTVEGVKALKEAIVAALP

SEQ ID NO: 6 - protein, 16 aa, synthetic construct
GGGGGSGGGGSGGGGS

SEQ ID NO: 7 - protein, 10 aa, synthetic construct
GGGGSGGGGS

SEQ ID NO: 8 - protein, 526 aa, synthetic construct
GRPFVEMYSEIPEIIHMTEGRELVIPCRVTSPNITVTLKKFPLDTLIPDGKRIIWDSRKGFIISNATYKEIGLLTCEATVNGHLYKTNYLTHRQTNTIIDVVLSPSHGIELSVGEKLVLNCTARTELNVGIDFNWEYPSSKHQHKKLVNRDLKTQSGSEMKKFLSTLTIDGVTRSDQGLYTCAASSGLMTKKNSTFVRVHEKPFVAFGSGMESLVEATVGERVRIPAKYLGYPPPEIKWYKNGIPLESNHTIKAGHVLTIMEVSERDTGNYTVILTNPISKEKQSHVVSLVVYVPPGPGDKTHTCPLCPAPELLGGPSVFLFPPKPKDTLMISRTPEVTCVVVDVSHEDPEVKFNWYVDGVEVHNAKTKPREEQYNSTYRVVSVLTVLHQDWLNGKEYKCKVSNKALPAPIEKTISKAKGQPREPQVYTLPPSRDELTKNQVSLTCLVKGFYPSDIAVEWESNGQPENNYKATPPVLDSDGSFFLYSKLTVDKSRWQQGNVFSCSVMHEALHNHYTQKSLSLSPGK